European Patent Specification EP 3 234 189 B1, published March 12, 2025. Title: Indel detection by amplicon analysis. Applicant: GeCo Aps. The sequence listing filed with the application follows.

SEQUENCE LISTING (133 sequences)

SEQ ID NO: 1 - DNA, 21 bp, Artificial Sequence
  consensus sequence of universal primer; n is any nucleotide
  misc_feature 1-3: /note="n is any nucleotide"
nnntgaccggcagcaaaattg

SEQ ID NO: 2 - DNA, 22 bp, Artificial Sequence
  FAMFOR extended with a 5' G; n is any nucleotide
  misc_feature 2..4: /note="n is any nucleotide"
gnnntgaccggcagcaaaattg

SEQ ID NO: 3 - DNA, 21 bp, Artificial Sequence
  FAMFOR primer
agctgaccggcagcaaaattg

SEQ ID NO: 4 - DNA, 22 bp, Artificial Sequence
  FAMFOR extended
gagctgaccggcagcaaaattg

SEQ ID NO: 5 - DNA, 18 bp, Artificial Sequence
  core sequence
tgaccggcagcaaaattg

SEQ ID NO: 6 - DNA, 21 bp, Artificial Sequence
  Variant 3
aaatgaccggcagcaaaattg

SEQ ID NO: 7 - DNA, 21 bp, Artificial Sequence
  Variant 4
aagtgaccggcagcaaaattg

SEQ ID NO: 8 - DNA, 21 bp, Artificial Sequence
  Variant 5
aactgaccggcagcaaaattg

SEQ ID NO: 9 - DNA, 21 bp, Artificial Sequence
  Variant 6
aattgaccggcagcaaaattg

SEQ ID NO: 10 - DNA, 21 bp, Artificial Sequence
  Variant 7
atatgaccggcagcaaaattg

SEQ ID NO: 11 - DNA, 21 bp, Artificial Sequence
  Variant 8
atgtgaccggcagcaaaattg

SEQ ID NO: 12 - DNA, 21 bp, Artificial Sequence
  Variant 9
atctgaccggcagcaaaattg

SEQ ID NO: 13 - DNA, 21 bp, Artificial Sequence
  Variant 10
atttgaccggcagcaaaattg

SEQ ID NO: 14 - DNA, 21 bp, Artificial Sequence
  Variant 11
acatgaccggcagcaaaattg

SEQ ID NO: 15 - DNA, 21 bp, Artificial Sequence
  Variant 12
acgtgaccggcagcaaaattg

SEQ ID NO: 16 - DNA, 21 bp, Artificial Sequence
  Variant 13
acctgaccggcagcaaaattg

SEQ ID NO: 17 - DNA, 21 bp, Artificial Sequence
  Variant 14
acttgaccggcagcaaaattg

SEQ ID NO: 18 - DNA, 21 bp, Artificial Sequence
  Variant 15
agatgaccggcagcaaaattg

SEQ ID NO: 19 - DNA, 21 bp, Artificial Sequence
  Variant 16
aggtgaccggcagcaaaattg

SEQ ID NO: 20 - DNA, 21 bp, Artificial Sequence
  Variant 17
agttgaccggcagcaaaattg

SEQ ID NO: 21 - DNA, 21 bp, Artificial Sequence
  Variant 18
taatgaccggcagcaaaattg

SEQ ID NO: 22 - DNA, 21 bp, Artificial Sequence
  Variant 19
tagtgaccggcagcaaaattg

SEQ ID NO: 23 - DNA, 21 bp, Artificial Sequence
  Variant 20
tactgaccggcagcaaaattg

SEQ ID NO: 24 - DNA, 21 bp, Artificial Sequence
  Variant 21
tattgaccggcagcaaaattg

SEQ ID NO: 25 - DNA, 21 bp, Artificial Sequence
  Variant 22
ttatgaccggcagcaaaattg

SEQ ID NO: 26 - DNA, 21 bp, Artificial Sequence
  Variant 23
ttgtgaccggcagcaaaattg

SEQ ID NO: 27 - DNA, 21 bp, Artificial Sequence
  Variant 24
ttctgaccggcagcaaaattg

SEQ ID NO: 28 - DNA, 21 bp, Artificial Sequence
  Variant 25
ttttgaccggcagcaaaattg

SEQ ID NO: 29 - DNA, 21 bp, Artificial Sequence
  Variant 26
tcatgaccggcagcaaaattg

SEQ ID NO: 30 - DNA, 21 bp, Artificial Sequence
  Variant 27
tcgtgaccggcagcaaaattg

SEQ ID NO: 31 - DNA, 21 bp, Artificial Sequence
  Variant 28
tcctgaccggcagcaaaattg

SEQ ID NO: 32 - DNA, 21 bp, Artificial Sequence
  Variant 29
tcttgaccggcagcaaaattg

SEQ ID NO: 33 - DNA, 21 bp, Artificial Sequence
  Variant 30
tgatgaccggcagcaaaattg

SEQ ID NO: 34 - DNA, 21 bp, Artificial Sequence
  Variant 31
tggtgaccggcagcaaaattg

SEQ ID NO: 35 - DNA, 21 bp, Artificial Sequence
  Variant 32
tgctgaccggcagcaaaattg

SEQ ID NO: 36 - DNA, 21 bp, Artificial Sequence
  Variant 33
tgttgaccggcagcaaaattg

SEQ ID NO: 37 - DNA, 21 bp, Artificial Sequence
  Variant 34
caatgaccggcagcaaaattg

SEQ ID NO: 38 - DNA, 21 bp, Artificial Sequence
  Variant 35
cagtgaccggcagcaaaattg

SEQ ID NO: 39 - DNA, 21 bp, Artificial Sequence
  Variant 36
cactgaccggcagcaaaattg

SEQ ID NO: 40 - DNA, 21 bp, Artificial Sequence
  Variant 37
cattgaccggcagcaaaattg

SEQ ID NO: 41 - DNA, 21 bp, Artificial Sequence
  Variant 38
ctatgaccggcagcaaaattg

SEQ ID NO: 42 - DNA, 21 bp, Artificial Sequence
  Variant 39
ctgtgaccggcagcaaaattg

SEQ ID NO: 43 - DNA, 21 bp, Artificial Sequence
  Variant 40
ctctgaccggcagcaaaattg

SEQ ID NO: 44 - DNA, 21 bp, Artificial Sequence
  Variant 41
ctttgaccggcagcaaaattg

SEQ ID NO: 45 - DNA, 21 bp, Artificial Sequence
  Variant 42
ccatgaccggcagcaaaattg

SEQ ID NO: 46 - DNA, 21 bp, Artificial Sequence
  Variant 43
ccgtgaccggcagcaaaattg

SEQ ID NO: 47 - DNA, 21 bp, Artificial Sequence
  Variant 44
ccctgaccggcagcaaaattg

SEQ ID NO: 48 - DNA, 21 bp, Artificial Sequence
  Variant 45
ccttgaccggcagcaaaattg

SEQ ID NO: 49 - DNA, 21 bp, Artificial Sequence
  Variant 46
cgatgaccggcagcaaaattg

SEQ ID NO: 50 - DNA, 21 bp, Artificial Sequence
  Variant 47
cggtgaccggcagcaaaattg

SEQ ID NO: 51 - DNA, 21 bp, Artificial Sequence
  Variant 48
cgctgaccggcagcaaaattg

SEQ ID NO: 52 - DNA, 21 bp, Artificial Sequence
  Variant 49
cgttgaccggcagcaaaattg

SEQ ID NO: 53 - DNA, 21 bp, Artificial Sequence
  Variant 50
gaatgaccggcagcaaaattg

SEQ ID NO: 54 - DNA, 21 bp, Artificial Sequence
  Variant 51
gagtgaccggcagcaaaattg

SEQ ID NO: 55 - DNA, 21 bp, Artificial Sequence
  Variant 52
gactgaccggcagcaaaattg

SEQ ID NO: 56 - DNA, 21 bp, Artificial Sequence
  Variant 53
gattgaccggcagcaaaattg

SEQ ID NO: 57 - DNA, 21 bp, Artificial Sequence
  Variant 54
gtatgaccggcagcaaaattg

SEQ ID NO: 58 - DNA, 21 bp, Artificial Sequence
  Variant 55
gtgtgaccggcagcaaaattg

SEQ ID NO: 59 - DNA, 21 bp, Artificial Sequence
  Variant 56
gtctgaccggcagcaaaattg

SEQ ID NO: 60 - DNA, 21 bp, Artificial Sequence
  Variant 57
gtttgaccggcagcaaaattg

SEQ ID NO: 61 - DNA, 21 bp, Artificial Sequence
  Variant 58
gcatgaccggcagcaaaattg

SEQ ID NO: 62 - DNA, 21 bp, Artificial Sequence
  Variant 59
gcgtgaccggcagcaaaattg

SEQ ID NO: 63 - DNA, 21 bp, Artificial Sequence
  Variant 60
gcctgaccggcagcaaaattg

SEQ ID NO: 64 - DNA, 21 bp, Artificial Sequence
  Variant 61
gcttgaccggcagcaaaattg

SEQ ID NO: 65 - DNA, 21 bp, Artificial Sequence
  Variant 62
ggatgaccggcagcaaaattg

SEQ ID NO: 66 - DNA, 21 bp, Artificial Sequence
  Variant 63
gggtgaccggcagcaaaattg

SEQ ID NO: 67 - DNA, 21 bp, Artificial Sequence
  Variant 64
ggctgaccggcagcaaaattg

SEQ ID NO: 68 - DNA, 21 bp, Artificial Sequence
  Variant 65
ggttgaccggcagcaaaattg

SEQ ID NO: 69 - DNA, 22 bp, Artificial Sequence
  Variant 66
gaaatgaccggcagcaaaattg

SEQ ID NO: 70 - DNA, 22 bp, Artificial Sequence
  Variant 67
gaagtgaccggcagcaaaattg

SEQ ID NO: 71 - DNA, 22 bp, Artificial Sequence
  Variant 68
gaactgaccggcagcaaaattg

SEQ ID NO: 72 - DNA, 22 bp, Artificial Sequence
  Variant 69
gaattgaccggcagcaaaattg

SEQ ID NO: 73 - DNA, 22 bp, Artificial Sequence
  Variant 70
gatatgaccggcagcaaaattg

SEQ ID NO: 74 - DNA, 22 bp, Artificial Sequence
  Variant 71
gatgtgaccggcagcaaaattg

SEQ ID NO: 75 - DNA, 22 bp, Artificial Sequence
  Variant 72
gatctgaccggcagcaaaattg

SEQ ID NO: 76 - DNA, 22 bp, Artificial Sequence
  Variant 73
gatttgaccggcagcaaaattg

SEQ ID NO: 77 - DNA, 22 bp, Artificial Sequence
  Variant 74
gacatgaccggcagcaaaattg

SEQ ID NO: 78 - DNA, 22 bp, Artificial Sequence
  Variant 75
gacgtgaccggcagcaaaattg

SEQ ID NO: 79 - DNA, 22 bp, Artificial Sequence
  Variant 76
gacctgaccggcagcaaaattg

SEQ ID NO: 80 - DNA, 22 bp, Artificial Sequence
  Variant 77
gacttgaccggcagcaaaattg

SEQ ID NO: 81 - DNA, 22 bp, Artificial Sequence
  Variant 78
gagatgaccggcagcaaaattg

SEQ ID NO: 82 - DNA, 22 bp, Artificial Sequence
  Variant 79
gaggtgaccggcagcaaaattg

SEQ ID NO: 83 - DNA, 22 bp, Artificial Sequence
  Variant 80
gagttgaccggcagcaaaattg

SEQ ID NO: 84 - DNA, 22 bp, Artificial Sequence
  Variant 81
gtaatgaccggcagcaaaattg

SEQ ID NO: 85 - DNA, 22 bp, Artificial Sequence
  Variant 82
gtagtgaccggcagcaaaattg

SEQ ID NO: 86 - DNA, 22 bp, Artificial Sequence
  Variant 83
gtactgaccggcagcaaaattg

SEQ ID NO: 87 - DNA, 22 bp, Artificial Sequence
  Variant 84
gtattgaccggcagcaaaattg

SEQ ID NO: 88 - DNA, 22 bp, Artificial Sequence
  Variant 85
gttatgaccggcagcaaaattg

SEQ ID NO: 89 - DNA, 22 bp, Artificial Sequence
  Variant 86
gttgtgaccggcagcaaaattg

SEQ ID NO: 90 - DNA, 22 bp, Artificial Sequence
  Variant 87
gttctgaccggcagcaaaattg

SEQ ID NO: 91 - DNA, 22 bp, Artificial Sequence
  Variant 88
gttttgaccggcagcaaaattg

SEQ ID NO: 92 - DNA, 22 bp, Artificial Sequence
  Variant 89
gtcatgaccggcagcaaaattg

SEQ ID NO: 93 - DNA, 22 bp, Artificial Sequence
  90
gtcgtgaccggcagcaaaattg

SEQ ID NO: 94 - DNA, 22 bp, Artificial Sequence
  Variant 91
gtcctgaccggcagcaaaattg

SEQ ID NO: 95 - DNA, 22 bp, Artificial Sequence
  Variant 92
gtcttgaccggcagcaaaattg

SEQ ID NO: 96 - DNA, 22 bp, Artificial Sequence
  Variant 93
gtgatgaccggcagcaaaattg

SEQ ID NO: 97 - DNA, 22 bp, Artificial Sequence
  Variant 94
gtggtgaccggcagcaaaattg

SEQ ID NO: 98 - DNA, 22 bp, Artificial Sequence
  Variant 95
gtgctgaccggcagcaaaattg

SEQ ID NO: 99 - DNA, 22 bp, Artificial Sequence
  Variant 96
gtgttgaccggcagcaaaattg

SEQ ID NO: 100 - DNA, 22 bp, Artificial Sequence
  Variant 97
gcaatgaccggcagcaaaattg

SEQ ID NO: 101 - DNA, 22 bp, Artificial Sequence
  Variant 98
gcagtgaccggcagcaaaattg

SEQ ID NO: 102 - DNA, 22 bp, Artificial Sequence
  Variant 99
gcactgaccggcagcaaaattg

SEQ ID NO: 103 - DNA, 22 bp, Artificial Sequence
  Variant 100
gcattgaccggcagcaaaattg

SEQ ID NO: 104 - DNA, 22 bp, Artificial Sequence
  Variant 101
gctatgaccggcagcaaaattg

SEQ ID NO: 105 - DNA, 22 bp, Artificial Sequence
  Variant 102
gctgtgaccggcagcaaaattg

SEQ ID NO: 106 - DNA, 22 bp, Artificial Sequence
  Variant 103
gctctgaccggcagcaaaattg

SEQ ID NO: 107 - DNA, 22 bp, Artificial Sequence
  Variant 104
gctttgaccggcagcaaaattg

SEQ ID NO: 108 - DNA, 22 bp, Artificial Sequence
  Variant 105
gccatgaccggcagcaaaattg

SEQ ID NO: 109 - DNA, 22 bp, Artificial Sequence
  Variant 106
gccgtgaccggcagcaaaattg

SEQ ID NO: 110 - DNA, 22 bp, Artificial Sequence
  Variant 107
gccctgaccggcagcaaaattg

SEQ ID NO: 111 - DNA, 22 bp, Artificial Sequence
  Variant 108
gccttgaccggcagcaaaattg

SEQ ID NO: 112 - DNA, 22 bp, Artificial Sequence
  Variant 109
gcgatgaccggcagcaaaattg

SEQ ID NO: 113 - DNA, 22 bp, Artificial Sequence
  Variant 110
gcggtgaccggcagcaaaattg

SEQ ID NO: 114 - DNA, 22 bp, Artificial Sequence
  Variant 111
gcgctgaccggcagcaaaattg

SEQ ID NO: 115 - DNA, 22 bp, Artificial Sequence
  Variant 112
gcgttgaccggcagcaaaattg

SEQ ID NO: 116 - DNA, 22 bp, Artificial Sequence
  Variant 113
ggaatgaccggcagcaaaattg

SEQ ID NO: 117 - DNA, 22 bp, Artificial Sequence
  Variant 114
ggagtgaccggcagcaaaattg

SEQ ID NO: 118 - DNA, 22 bp, Artificial Sequence
  Variant 115
ggactgaccggcagcaaaattg

SEQ ID NO: 119 - DNA, 22 bp, Artificial Sequence
  Variant 116
ggattgaccggcagcaaaattg

SEQ ID NO: 120 - DNA, 22 bp, Artificial Sequence
  Variant 117
ggtatgaccggcagcaaaattg

SEQ ID NO: 121 - DNA, 22 bp, Artificial Sequence
  Variant 118
ggtgtgaccggcagcaaaattg

SEQ ID NO: 122 - DNA, 22 bp, Artificial Sequence
  Variant 119
ggtctgaccggcagcaaaattg

SEQ ID NO: 123 - DNA, 22 bp, Artificial Sequence
  Variant 120
ggtttgaccggcagcaaaattg

SEQ ID NO: 124 - DNA, 22 bp, Artificial Sequence
  Variant 121
ggcatgaccggcagcaaaattg

SEQ ID NO: 125 - DNA, 22 bp, Artificial Sequence
  Variant 122
ggcgtgaccggcagcaaaattg

SEQ ID NO: 126 - DNA, 22 bp, Artificial Sequence
  Variant 123
ggcctgaccggcagcaaaattg

SEQ ID NO: 127 - DNA, 22 bp, Artificial Sequence
  Variant 124
ggcttgaccggcagcaaaattg

SEQ ID NO: 128 - DNA, 22 bp, Artificial Sequence
  Variant 125
gggatgaccggcagcaaaattg

SEQ ID NO: 129 - DNA, 22 bp, Artificial Sequence
  Variant 126
ggggtgaccggcagcaaaattg

SEQ ID NO: 130 - DNA, 22 bp, Artificial Sequence
  Variant 127
gggctgaccggcagcaaaattg

SEQ ID NO: 131 - DNA, 22 bp, Artificial Sequence
  Variant 128
gggttgaccggcagcaaaattg

SEQ ID NO: 132 - DNA, 47 bp, Artificial Sequence
  CXCR4 forward extension primer
  misc_binding 1..22: /note="adaptamer tail"
  primer_bind 23..47: /PCR_conditions="binds to target"
gagctgaccggcagcaaaattgcaacctctacagcagtgtcctcatc

SEQ ID NO: 133 - DNA, 22 bp, Artificial Sequence
  CXCR4 reverse primer
ggagtgtgacagcttggagatg